European Patent Application EP 4 800 110 A1, published September 2, 2026. Title: Gapmer antisense oligonucleotide for targeting the RHO gene. Applicant: Eberhard Karls Universität Tübingen - Medizinische Fakultät. Application EP. The sequence listing filed with the application follows.

SEQUENCE LISTING (37 sequences)

SEQ ID NO: 1 - DNA, 31 bp, synthetic construct
  source 1..31: mol_type = other DNA
tgggtgggagcagccrcgggtcagccacaag

SEQ ID NO: 2 - RNA, 31 nt, synthetic construct
  source 1..31: mol_type = other RNA
tgggtgggagcagccrcgggtcagccacaag

SEQ ID NO: 3 - DNA, 16 bp, synthetic construct
  source 1..16: mol_type = other DNA
gctgacccgtggctgc

SEQ ID NO: 4 - DNA, 16 bp, synthetic construct
  source 1..16: mol_type = other DNA
ggctgacccgtggctg

SEQ ID NO: 5 - DNA, 16 bp, synthetic construct
  source 1..16: mol_type = other DNA
ggctgacccgtggctg

SEQ ID NO: 6 - DNA, 16 bp, synthetic construct
  source 1..16: mol_type = other DNA
gcggctgctcccaccc

SEQ ID NO: 7 - DNA, 16 bp, synthetic construct
  source 1..16: mol_type = other DNA
cgtggctgctcccacc

SEQ ID NO: 8 - DNA, 16 bp, synthetic construct
  source 1..16: mol_type = other DNA
acccgtggctgctccc

SEQ ID NO: 9 - DNA, 16 bp, synthetic construct
  source 1..16: mol_type = other DNA
ctgacccgtggctgct

SEQ ID NO: 10 - DNA, 16 bp, synthetic construct
  source 1..16: mol_type = other DNA
cttgtggctgacccgt

SEQ ID NO: 11 - DNA, 16 bp, synthetic construct
  source 1..16: mol_type = other DNA
ttgtggctgacccgtg

SEQ ID NO: 12 - DNA, 16 bp, synthetic construct
  source 1..16: mol_type = other DNA
gtggctgacccgtggc

SEQ ID NO: 13 - DNA, 16 bp, synthetic construct
  source 1..16: mol_type = other DNA
tggctgacccgtggct

SEQ ID NO: 14 - DNA, 16 bp, synthetic construct
  source 1..16: mol_type = other DNA
gacccgtggctgctcc

SEQ ID NO: 15 - DNA, 16 bp, synthetic construct
  source 1..16: mol_type = other DNA
cccgtggctgctccca

SEQ ID NO: 16 - DNA, 16 bp, synthetic construct
  source 1..16: mol_type = other DNA
ccgtggctgctcccac

SEQ ID NO: 17 - DNA, 16 bp, synthetic construct
  source 1..16: mol_type = other DNA
gtggctgctcccaccc

SEQ ID NO: 18 - DNA, 16 bp, synthetic construct
  source 1..16: mol_type = other DNA
tggctgctcccaccca

SEQ ID NO: 19 - DNA, 16 bp, synthetic construct
  source 1..16: mol_type = other DNA
tgacccgcggctgctc

SEQ ID NO: 20 - DNA, 16 bp, synthetic construct
  source 1..16: mol_type = other DNA
tgtggctgacccgcgg

SEQ ID NO: 21 - DNA, 16 bp, synthetic construct
  source 1..16: mol_type = other DNA
cgcggctgctcccacc

SEQ ID NO: 22 - DNA, 16 bp, synthetic construct
  source 1..16: mol_type = other DNA
acccgcggctgctccc

SEQ ID NO: 23 - DNA, 16 bp, synthetic construct
  source 1..16: mol_type = other DNA
gctgacccgcggctgc

SEQ ID NO: 24 - DNA, 16 bp, synthetic construct
  source 1..16: mol_type = other DNA
ctgacccgcggctgct

SEQ ID NO: 25 - DNA, 16 bp, synthetic construct
  source 1..16: mol_type = other DNA
cttgtggctgacccgc

SEQ ID NO: 26 - DNA, 16 bp, synthetic construct
  source 1..16: mol_type = other DNA
ttgtggctgacccgcg

SEQ ID NO: 27 - DNA, 16 bp, synthetic construct
  source 1..16: mol_type = other DNA
gtggctgacccgcggc

SEQ ID NO: 28 - DNA, 16 bp, synthetic construct
  source 1..16: mol_type = other DNA
tggctgacccgcggct

SEQ ID NO: 29 - DNA, 16 bp, synthetic construct
  source 1..16: mol_type = other DNA
ggctgacccgcggctg

SEQ ID NO: 30 - DNA, 16 bp, synthetic construct
  source 1..16: mol_type = other DNA
gacccgcggctgctcc

SEQ ID NO: 31 - DNA, 16 bp, synthetic construct
  source 1..16: mol_type = other DNA
ccgcggctgctcccac

SEQ ID NO: 32 - DNA, 16 bp, synthetic construct
  source 1..16: mol_type = other DNA
cggctgctcccaccca

SEQ ID NO: 33 - DNA, 10 bp, synthetic construct
  source 1..10: mol_type = other DNA
gacccgtggc

SEQ ID NO: 34 - DNA, 10 bp, synthetic construct
  source 1..10: mol_type = other DNA
tgacccgtgg

SEQ ID NO: 35 - DNA, 10 bp, synthetic construct
  source 1..10: mol_type = other DNA
gcggctgctc

SEQ ID NO: 36 - DNA, 10 bp, synthetic construct
  source 1..10: mol_type = other DNA
gctgctccca

SEQ ID NO: 37 - skipped